European Patent Application EP 4 296 357 A1, published December 27, 2023. Title: Novel anti PAD4 antibody. Applicant: Mitsubishi Tanabe Pharma Corporation Pharma Foods International Co., Ltd. The sequence listing filed with the application follows.

SEQUENCE LISTING (40 sequences)

SEQ ID NO: 1 - protein, 5 aa, Artificial Sequence
  HCDR
TYAMG

SEQ ID NO: 2 - protein, 17 aa, Artificial Sequence
  HCDR
  misc_difference (11)..(11): Tyr, Thr or Ile
  misc_difference (12)..(12): Gly, Ser or Pro
  misc_difference (13)..(13): Thr, Val Tyr or Pro
  misc_difference (14)..(14): Pro or Asn
  misc_difference (15)..(15): Tyr, Ala, Gln or Leu
  misc_difference (17)..(17): Gly, Thr or Ser
AIRNDGSWTGXXXXXKX

SEQ ID NO: 3 - protein, 13 aa, Artificial Sequence
  HCDR
  misc_difference (1)..(1): Ala or Gly
XKYTGSSGGSIGA

SEQ ID NO: 4 - protein, 10 aa, Artificial Sequence
  LCDR
SGGNRNYYYG

SEQ ID NO: 5 - protein, 7 aa, Artificial Sequence
  LCDR
ANDKRPS

SEQ ID NO: 6 - protein, 9 aa, Artificial Sequence
  LCDR
  misc_difference (4)..(4): Thr, Leu or Tyr
GTAXTGKYV

SEQ ID NO: 7 - protein, 17 aa, Artificial Sequence
  HCDR
AIRNDGSWTGYGTPYKT

SEQ ID NO: 8 - protein, 17 aa, Artificial Sequence
  HCDR
AIRNDGSWTGTSVNAKT

SEQ ID NO: 9 - protein, 17 aa, Artificial Sequence
  HCDR
AIRNDGSWTGIGYNQKS

SEQ ID NO: 10 - protein, 17 aa, Artificial Sequence
  HCDR
AIRNDGSWTGYPPPLKG

SEQ ID NO: 11 - protein, 13 aa, Artificial Sequence
  HCDR
AKYTGSSGGSIGA

SEQ ID NO: 12 - protein, 13 aa, Artificial Sequence
  HCDR
GKYTGSSGGSIGA

SEQ ID NO: 13 - protein, 9 aa, Artificial Sequence
  LCDR
GTATTGKYV

SEQ ID NO: 14 - protein, 9 aa, Artificial Sequence
  LCDR
GTALTGKYV

SEQ ID NO: 15 - protein, 9 aa, Artificial Sequence
  LCDR
GTAYTGKYV

SEQ ID NO: 16 - protein, 450 aa, Artificial Sequence
  Antibody heavy chain
EVQLLESGGGLVQPGGSLRLSCAASGFTFSTYAMGWVRQAPGKGLEFVAAIRNDGSWTGYGTPYKTRFTISRDNSKNTLYLQMSSLRAEDTAVYYCAKYTGSSGGSIGAWGQGTLVTVSSASTKGPSVFPLAPSSKSTSGGTAALGCLVKDYFPEPVTVSWNSGALTSGVHTFPAVLQSSGLYSLSSVVTVPSSSLGTQTYICNVNHKPSNTKVDKKVEPKSCDKTHTCPPCPAPELLGGPSVFLFPPKPKDTLMISRTPEVTCVVVDVSHEDPEVKFNWYVDGVEVHNAKTKPREEQYNSTYRVVSVLTVLHQDWLNGKEYKCKVSNKALPAPIEKTISKAKGQPREPQVYTLPPSRDELTKNQVSLTCLVKGFYPSDIAVEWESNGQPENNYKTTPPVLDSDGSFFLYSKLTVDKSRWQQGNVFSCSVMHEALHNHYTQKSLSLSPGK

SEQ ID NO: 17 - protein, 210 aa, Artificial Sequence
  Antibody light chain
SYELTQPPSVSVSPGQTARITCSGGNRNYYYGWYQQKPGQAPVTVIYANDKRPSGIPERFSGSNSGSTTTLTISGVQAEDEADYYCGTATTGKYVFGGGTKLTVLGQPKAAPSVTLFPPSSEELQANKATLVCLISDFYPGAVTVAWKADSSPVKAGVETTTPSKQSNNKYAASSYLSLTPEQWKSHRSYSCQVTHEGSTVEKTVAPTEC

SEQ ID NO: 18 - protein, 450 aa, Artificial Sequence
  Antibody heavy chain
EVQLLESGGGLVQPGGSLRLSCAASGFTFSTYAMGWVRQAPGKGLEFVAAIRNDGSWTGTSVNAKTRFTISRDNSKNTLYLQMSSLRAEDTAVYYCAKYTGSSGGSIGAWGQGTLVTVSSASTKGPSVFPLAPSSKSTSGGTAALGCLVKDYFPEPVTVSWNSGALTSGVHTFPAVLQSSGLYSLSSVVTVPSSSLGTQTYICNVNHKPSNTKVDKKVEPKSCDKTHTCPPCPAPELLGGPSVFLFPPKPKDTLMISRTPEVTCVVVDVSHEDPEVKFNWYVDGVEVHNAKTKPREEQYNSTYRVVSVLTVLHQDWLNGKEYKCKVSNKALPAPIEKTISKAKGQPREPQVYTLPPSRDELTKNQVSLTCLVKGFYPSDIAVEWESNGQPENNYKTTPPVLDSDGSFFLYSKLTVDKSRWQQGNVFSCSVMHEALHNHYTQKSLSLSPGK

SEQ ID NO: 19 - protein, 210 aa, Artificial Sequence; identical to SEQ ID NO: 17
  Antibody light chain

SEQ ID NO: 20 - protein, 450 aa, Artificial Sequence
  Antibody heavy chain
EVQLLESGGGLVQPGGSLRLSCAASGFTFSTYAMGWVRQAPGKGLEFVAAIRNDGSWTGIGYNQKSRFTISRDNSKNTLYLQMSSLRAEDTAVYYCGKYTGSSGGSIGAWGQGTLVTVSSASTKGPSVFPLAPSSKSTSGGTAALGCLVKDYFPEPVTVSWNSGALTSGVHTFPAVLQSSGLYSLSSVVTVPSSSLGTQTYICNVNHKPSNTKVDKKVEPKSCDKTHTCPPCPAPELLGGPSVFLFPPKPKDTLMISRTPEVTCVVVDVSHEDPEVKFNWYVDGVEVHNAKTKPREEQYNSTYRVVSVLTVLHQDWLNGKEYKCKVSNKALPAPIEKTISKAKGQPREPQVYTLPPSRDELTKNQVSLTCLVKGFYPSDIAVEWESNGQPENNYKTTPPVLDSDGSFFLYSKLTVDKSRWQQGNVFSCSVMHEALHNHYTQKSLSLSPGK

SEQ ID NO: 21 - protein, 210 aa, Artificial Sequence
  Antibody light chain
SYELTQPPSVSVSPGQTARITCSGGNRNYYYGWYQQKPGQAPVTVIYANDKRPSGIPERFSGSNSGSTTTLTISGVQAEDEADYYCGTALTGKYVFGGGTKLTVLGQPKAAPSVTLFPPSSEELQANKATLVCLISDFYPGAVTVAWKADSSPVKAGVETTTPSKQSNNKYAASSYLSLTPEQWKSHRSYSCQVTHEGSTVEKTVAPTEC

SEQ ID NO: 22 - protein, 450 aa, Artificial Sequence
  Antibody heavy chain
EVQLLESGGGLVQPGGSLRLSCAASGFTFSTYAMGWVRQAPGKGLEFVAAIRNDGSWTGYPPPLKGRFTISRDNSKNTLYLQMSSLRAEDTAVYYCAKYTGSSGGSIGAWGQGTLVTVSSASTKGPSVFPLAPSSKSTSGGTAALGCLVKDYFPEPVTVSWNSGALTSGVHTFPAVLQSSGLYSLSSVVTVPSSSLGTQTYICNVNHKPSNTKVDKKVEPKSCDKTHTCPPCPAPELLGGPSVFLFPPKPKDTLMISRTPEVTCVVVDVSHEDPEVKFNWYVDGVEVHNAKTKPREEQYNSTYRVVSVLTVLHQDWLNGKEYKCKVSNKALPAPIEKTISKAKGQPREPQVYTLPPSRDELTKNQVSLTCLVKGFYPSDIAVEWESNGQPENNYKTTPPVLDSDGSFFLYSKLTVDKSRWQQGNVFSCSVMHEALHNHYTQKSLSLSPGK

SEQ ID NO: 23 - protein, 210 aa, Artificial Sequence
  Antibody light chain
SYELTQPPSVSVSPGQTARITCSGGNRNYYYGWYQQKPGQAPVTVIYANDKRPSGIPERFSGSNSGSTTTLTISGVQAEDEADYYCGTAYTGKYVFGGGTKLTVLGQPKAAPSVTLFPPSSEELQANKATLVCLISDFYPGAVTVAWKADSSPVKAGVETTTPSKQSNNKYAASSYLSLTPEQWKSHRSYSCQVTHEGSTVEKTVAPTEC

SEQ ID NO: 24 - protein, 17 aa, Artificial Sequence
  HCDR
AIRNDGSWTGYGAAVKG

SEQ ID NO: 25 - protein, 9 aa, Artificial Sequence
  LCDR
GTADTGKYV

SEQ ID NO: 26 - protein, 450 aa, Artificial Sequence
  Antibody heavy chain
EVQLLESGGGLVQPGGSLRLSCAASGFTFSTYAMGWVRQAPGKGLEFVAAIRNDGSWTGYGAAVKGRFTISRDNSKNTLYLQMNSLRAEDTAVYYCAKYTGSSGGSIGAWGQGTLVTVSSASTKGPSVFPLAPSSKSTSGGTAALGCLVKDYFPEPVTVSWNSGALTSGVHTFPAVLQSSGLYSLSSVVTVPSSSLGTQTYICNVNHKPSNTKVDKKVEPKSCDKTHTCPPCPAPELLGGPSVFLFPPKPKDTLMISRTPEVTCVVVDVSHEDPEVKFNWYVDGVEVHNAKTKPREEQYNSTYRVVSVLTVLHQDWLNGKEYKCKVSNKALPAPIEKTISKAKGQPREPQVYTLPPSRDELTKNQVSLTCLVKGFYPSDIAVEWESNGQPENNYKTTPPVLDSDGSFFLYSKLTVDKSRWQQGNVFSCSVMHEALHNHYTQKSLSLSPGK

SEQ ID NO: 27 - protein, 210 aa, Artificial Sequence
  Antibody light chain
SYELTQPPSVSVSPGQTARITCSGGNRNYYYGWYQQKPGQAPVTVIYANDKRPSGIPERFSGSNSGSTTTLTISGVQAEDEADYYCGTADTGKYVFGGGTKLTVLGQPKAAPSVTLFPPSSEELQANKATLVCLISDFYPGAVTVAWKADSSPVKAGVETTTPSKQSNNKYAASSYLSLTPEQWKSHRSYSCQVTHEGSTVEKTVAPTEC

SEQ ID NO: 28 - protein, 450 aa, Artificial Sequence
  Antibody heavy chain
EVQLLESGGGLVQPGGSLRLSCAASGFTFSTYAMGWVRQAPGKGLEFVAAIRNDGSWTGYGAAVKGRFTISRDNSKNTLYLQMSSLRAEDTAVYYCAKYTGSSGGSIGAWGQGTLVTVSSASTKGPSVFPLAPSSKSTSGGTAALGCLVKDYFPEPVTVSWNSGALTSGVHTFPAVLQSSGLYSLSSVVTVPSSSLGTQTYICNVNHKPSNTKVDKKVEPKSCDKTHTCPPCPAPELLGGPSVFLFPPKPKDTLMISRTPEVTCVVVDVSHEDPEVKFNWYVDGVEVHNAKTKPREEQYNSTYRVVSVLTVLHQDWLNGKEYKCKVSNKALPAPIEKTISKAKGQPREPQVYTLPPSRDELTKNQVSLTCLVKGFYPSDIAVEWESNGQPENNYKTTPPVLDSDGSFFLYSKLTVDKSRWQQGNVFSCSVMHEALHNHYTQKSLSLSPGK

SEQ ID NO: 29 - protein, 663 aa, Homo sapiens
MAQGTLIRVTPEQPTHAVCVLGTLTQLDICSSAPEDCTSFSINASPGVVVDIAHGPPAKKKSTGSSTWPLDPGVEVTLTMKVASGSTGDQKVQISYYGPKTPPVKALLYLTGVEISLCADITRTGKVKPTRAVKDQRTWTWGPCGQGAILLVNCDRDNLESSAMDCEDDEVLDSEDLQDMSLMTLSTKTPKDFFTNHTLVLHVARSEMDKVRVFQATRGKLSSKCSVVLGPKWPSHYLMVPGGKHNMDFYVEALAFPDTDFPGLITLTISLLDTSNLELPEAVVFQDSVVFRVAPWIMTPNTQPPQEVYACSIFENEDFLKSVTTLAMKAKCKLTICPEEENMDDQWMQDEMEIGYIQAPHKTLPVVFDSPRNRGLKEFPIKRVMGPDFGYVTRGPQTGGISGLDSFGNLEVSPPVTVRGKEYPLGRILFGDSCYPSNDSRQMHQALQDFLSAQQVQAPVKLYSDWLSVGHVDEFLSFVPAPDRKGFRLLLASPRSCYKLFQEQQNEGHGEALLFEGIKKKKQQKIKNILSNKTLREHNSFVERCIDWNRELLKRELGLAESDIIDIPQLFKLKEFSKAEAFFPNMVNMLVLGKHLGIPKPFGPVINGRCCLEEKVCSLLEPLGLQCTFINDFFTYHIRHGEVHCGTNVRRKPFSFKWWNMVP

SEQ ID NO: 30 - DNA, 1353 bp, Artificial Sequence
  Antibody heavy chain
gaggtgcagctgttggagtctgggggaggactggtgcagcctggcggaagcctgagactgtcttgtgccgccagcggcttcaccttcagcacctatgccatgggctgggtgcgccaggcccctggaaagggcctggaatttgtggccgccatccggaacgatggcagctggacaggatatggcgccgctgtgaagggccggttcaccatcagccgggacaacagcaagaacaccctgtacctgcagatgaacagcctgcgggccgaggacaccgccgtgtactactgtgccaagtacaccggcagcagcggcggctctattggagcttggggacagggaaccctggtcaccgtctcctcagcctctacaaagggccccagcgtgttccctctggcccctagcagcaagagcacatctggcggaacagccgccctgggctgcctcgtgaaggactactttcccgagcccgtgaccgtgtcctggaactctggcgctctgacaagcggcgtgcacacctttccagccgtgctgcagagcagcggcctgtactctctgagcagcgtcgtgacagtgcccagcagctctctgggcacccagacctacatctgcaacgtgaaccacaagcccagcaacaccaaggtggacaagaaggtggaacccaagagctgcgacaagacccacacctgtcccccttgtcctgcccccgaactgctgggaggcccttccgtgttcctgttccccccaaagcccaaggacaccctgatgatcagccggacccccgaagtgacctgcgtggtggtggatgtgtcccacgaggaccctgaagtgaagttcaattggtacgtggacggcgtggaagtgcacaacgccaagaccaagcctagagaggaacagtacaacagcacctaccgggtggtgtccgtgctgacagtgctgcaccaggactggctgaacggcaaagagtacaagtgcaaggtgtccaacaaggccctgcctgcccccatcgagaaaaccatcagcaaggccaagggccagccccgcgaaccccaggtgtacacactgcccccaagcagggacgagctgaccaagaaccaggtgtccctgacctgtctcgtgaaaggcttctacccctccgatatcgccgtggaatgggagagcaacggccagcccgagaacaactacaagaccaccccccctgtgctggacagcgacggctcattcttcctgtacagcaagctgaccgtggacaagtcccggtggcagcagggcaacgtgttcagctgcagcgtgatgcacgaggccctgcacaaccactacacccagaagtccctgagcctgagccccggcaaatag

SEQ ID NO: 31 - DNA, 633 bp, Artificial Sequence
  Antibody light chain
agctatgagctgactcagccaccctcggtgtcagtgtccccaggacagacggccaggatcacctgctccggggggaataggaactactactatggctggtaccagcagaagccaggccaggcccctgtgaccgtgatatatgctaacgacaagagaccctcgggaatccctgagcgattctctggctccaactcagggtcaacaaccacgttgaccatcagtggagtccaggcagaagatgaggctgactattactgtgggaccgcagacaccgggaagtatgtattcggcggagggaccaagctgaccgtcctgggtcagcccaaggctgccccctcggtcactctgttcccgccctcctctgaggagcttcaagccaacaaggccacactggtgtgtctcataagtgacttctacccgggagccgtgacagtggcctggaaggcagatagcagccccgtcaaggcgggagtggagaccaccacaccctccaaacaaagcaacaacaagtacgcggccagcagctatctgagcctgacgcctgagcagtggaagtcccacagaagctacagctgccaggtcacgcatgaagggagcaccgtggagaagacagtggcccctacagaatgttag

SEQ ID NO: 32 - DNA, 1353 bp, Artificial Sequence
  Antibody heavy chain
gaagtacagctgcttgagagtggcggagggttggtccaacctggtgggtccttacgactgagctgtgcagcatctggcttcaccttcagcacctatgcgatgggatgggttcgtcaggctcccggtaaaggcctggagtttgtggctgccatacgcaatgatgggtcttggactgggtatgggactccttataaaactcggtttacgatctcaagggacaactccaagaataccctctatctccagatgtcttctctaagagccgaagacacagccgtgtactactgcgccaagtacactgggtcaagtggaggctcgattggcgcatggggtcagggaacactggtcacagtgtccagcgcctctacaaagggccccagcgtgttccctctggcccctagcagcaagagcacatctggcggaacagccgccctgggctgcctcgtgaaggactactttcccgagcccgtgaccgtgtcctggaactctggcgctctgacaagcggcgtgcacacctttccagccgtgctgcagagcagcggcctgtactctctgagcagcgtcgtgacagtgcccagcagctctctgggcacccagacctacatctgcaacgtgaaccacaagcccagcaacaccaaggtggacaagaaggtggaacccaagagctgcgacaagacccacacctgtcccccttgtcctgcccccgaactgctgggaggcccttccgtgttcctgttccccccaaagcccaaggacaccctgatgatcagccggacccccgaagtgacctgcgtggtggtggatgtgtcccacgaggaccctgaagtgaagttcaattggtacgtggacggcgtggaagtgcacaacgccaagaccaagcctagagaggaacagtacaacagcacctaccgggtggtgtccgtgctgacagtgctgcaccaggactggctgaacggcaaagagtacaagtgcaaggtgtccaacaaggccctgcctgcccccatcgagaaaaccatcagcaaggccaagggccagccccgcgaaccccaggtgtacacactgcccccaagcagggacgagctgaccaagaaccaggtgtccctgacctgtctcgtgaaaggcttctacccctccgatatcgccgtggaatgggagagcaacggccagcccgagaacaactacaagaccaccccccctgtgctggacagcgacggctcattcttcctgtacagcaagctgaccgtggacaagtcccggtggcagcagggcaacgtgttcagctgcagcgtgatgcacgaggccctgcacaaccactacacccagaagtccctgagcctgagccccggcaaatga

SEQ ID NO: 33 - DNA, 633 bp, Artificial Sequence
  Antibody light chain
tcgtatgagctgacacaacctccctcagtgtccgtaagtccaggacagactgcgagaatcacctgctctggaggcaatcgcaactactactatgggtggtatcagcagaaacccggacaagctcctgtgaccgtcatctatgccaacgacaaacggccatcaggcattccggagaggttcagcggtagcaattccgggtctaccaccactctcacgataagtggggttcaggctgaagatgaagccgactactactgtggcacagcaaccacaggcaagtacgtgtttggtggaggcactaagctgacagtccttggtcagcccaaggctgccccctcggtcactctgttcccgccctcctctgaggagcttcaagccaacaaggccacactggtgtgtctcataagtgacttctacccgggagccgtgacagtggcctggaaggcagatagcagccccgtcaaggcgggagtggagaccaccacaccctccaaacaaagcaacaacaagtacgcggccagcagctatctgagcctgacgcctgagcagtggaagtcccacagaagctacagctgccaggtcacgcatgaagggagcaccgtggagaagacagtggcccctacagaatgttag

SEQ ID NO: 34 - DNA, 1353 bp, Artificial Sequence
  Antibody heavy chain
gaagtacagctgcttgagagtggcggagggttggtccaacctggtgggtccttacgactgagctgtgcagcatctggcttcaccttcagcacctatgcgatgggatgggttcgtcaggctcccggtaaaggcctggagtttgtggctgccatacgcaatgatgggtcttggactgggactagtgtgaatgctaaaacgcggtttacgatctcaagggacaactccaagaataccctctatctccagatgtcttctctaagagccgaagacacagccgtgtactactgcgccaagtacactgggtcaagtggaggctcgattggcgcatggggtcagggaacactggtcacagtgtccagcgcctctacaaagggccccagcgtgttccctctggcccctagcagcaagagcacatctggcggaacagccgccctgggctgcctcgtgaaggactactttcccgagcccgtgaccgtgtcctggaactctggcgctctgacaagcggcgtgcacacctttccagccgtgctgcagagcagcggcctgtactctctgagcagcgtcgtgacagtgcccagcagctctctgggcacccagacctacatctgcaacgtgaaccacaagcccagcaacaccaaggtggacaagaaggtggaacccaagagctgcgacaagacccacacctgtcccccttgtcctgcccccgaactgctgggaggcccttccgtgttcctgttccccccaaagcccaaggacaccctgatgatcagccggacccccgaagtgacctgcgtggtggtggatgtgtcccacgaggaccctgaagtgaagttcaattggtacgtggacggcgtggaagtgcacaacgccaagaccaagcctagagaggaacagtacaacagcacctaccgggtggtgtccgtgctgacagtgctgcaccaggactggctgaacggcaaagagtacaagtgcaaggtgtccaacaaggccctgcctgcccccatcgagaaaaccatcagcaaggccaagggccagccccgcgaaccccaggtgtacacactgcccccaagcagggacgagctgaccaagaaccaggtgtccctgacctgtctcgtgaaaggcttctacccctccgatatcgccgtggaatgggagagcaacggccagcccgagaacaactacaagaccaccccccctgtgctggacagcgacggctcattcttcctgtacagcaagctgaccgtggacaagtcccggtggcagcagggcaacgtgttcagctgcagcgtgatgcacgaggccctgcacaaccactacacccagaagtccctgagcctgagccccggcaaatga

SEQ ID NO: 35 - DNA, 633 bp, Artificial Sequence; identical to SEQ ID NO: 33
  Antibody light chain

SEQ ID NO: 36 - DNA, 1353 bp, Artificial Sequence
  Antibody heavy chain
gaagtacagctgcttgagagtggcggagggttggtccaacctggtgggtccttacgactgagctgtgcagcatctggcttcaccttcagcacctatgcgatgggatgggttcgtcaggctcccggtaaaggcctggagtttgtggctgccatacgcaatgatgggtcttggactgggataggttataatcagaaatctcggtttacgatctcaagggacaactccaagaataccctctatctccagatgtcttctctaagagccgaagacacagccgtgtactactgcggtaagtacactgggtcaagtggaggctcgattggcgcatggggtcagggaacactggtcacagtgtccagcgcctctacaaagggccccagcgtgttccctctggcccctagcagcaagagcacatctggcggaacagccgccctgggctgcctcgtgaaggactactttcccgagcccgtgaccgtgtcctggaactctggcgctctgacaagcggcgtgcacacctttccagccgtgctgcagagcagcggcctgtactctctgagcagcgtcgtgacagtgcccagcagctctctgggcacccagacctacatctgcaacgtgaaccacaagcccagcaacaccaaggtggacaagaaggtggaacccaagagctgcgacaagacccacacctgtcccccttgtcctgcccccgaactgctgggaggcccttccgtgttcctgttccccccaaagcccaaggacaccctgatgatcagccggacccccgaagtgacctgcgtggtggtggatgtgtcccacgaggaccctgaagtgaagttcaattggtacgtggacggcgtggaagtgcacaacgccaagaccaagcctagagaggaacagtacaacagcacctaccgggtggtgtccgtgctgacagtgctgcaccaggactggctgaacggcaaagagtacaagtgcaaggtgtccaacaaggccctgcctgcccccatcgagaaaaccatcagcaaggccaagggccagccccgcgaaccccaggtgtacacactgcccccaagcagggacgagctgaccaagaaccaggtgtccctgacctgtctcgtgaaaggcttctacccctccgatatcgccgtggaatgggagagcaacggccagcccgagaacaactacaagaccaccccccctgtgctggacagcgacggctcattcttcctgtacagcaagctgaccgtggacaagtcccggtggcagcagggcaacgtgttcagctgcagcgtgatgcacgaggccctgcacaaccactacacccagaagtccctgagcctgagccccggcaaatga

SEQ ID NO: 37 - DNA, 633 bp, Artificial Sequence
  Antibody light chain
tcgtatgagctgacacaacctccctcagtgtccgtaagtccaggacagactgcgagaatcacctgctctggaggcaatcgcaactactactatgggtggtatcagcagaaacccggacaagctcctgtgaccgtcatctatgccaacgacaaacggccatcaggcattccggagaggttcagcggtagcaattccgggtctaccaccactctcacgataagtggggttcaggctgaagatgaagccgactactactgtggcacagcactcacaggcaagtacgtgtttggtggaggcactaagctgacagtccttggtcagcccaaggctgccccctcggtcactctgttcccgccctcctctgaggagcttcaagccaacaaggccacactggtgtgtctcataagtgacttctacccgggagccgtgacagtggcctggaaggcagatagcagccccgtcaaggcgggagtggagaccaccacaccctccaaacaaagcaacaacaagtacgcggccagcagctatctgagcctgacgcctgagcagtggaagtcccacagaagctacagctgccaggtcacgcatgaagggagcaccgtggagaagacagtggcccctacagaatgttag

SEQ ID NO: 38 - DNA, 1353 bp, Artificial Sequence
  Antibody heavy chain
gaagtacagctgcttgagagtggcggagggttggtccaacctggtgggtccttacgactgagctgtgcagcatctggcttcaccttcagcacctatgcgatgggatgggttcgtcaggctcccggtaaaggcctggagtttgtggctgccatacgcaatgatgggtcttggactgggtatcctcctcctcttaaaggtcggtttacgatctcaagggacaactccaagaataccctctatctccagatgtcttctctaagagccgaagacacagccgtgtactactgcgccaagtacactgggtcaagtggaggctcgattggcgcatggggtcagggaacactggtcacagtgtccagcgcctctacaaagggccccagcgtgttccctctggcccctagcagcaagagcacatctggcggaacagccgccctgggctgcctcgtgaaggactactttcccgagcccgtgaccgtgtcctggaactctggcgctctgacaagcggcgtgcacacctttccagccgtgctgcagagcagcggcctgtactctctgagcagcgtcgtgacagtgcccagcagctctctgggcacccagacctacatctgcaacgtgaaccacaagcccagcaacaccaaggtggacaagaaggtggaacccaagagctgcgacaagacccacacctgtcccccttgtcctgcccccgaactgctgggaggcccttccgtgttcctgttccccccaaagcccaaggacaccctgatgatcagccggacccccgaagtgacctgcgtggtggtggatgtgtcccacgaggaccctgaagtgaagttcaattggtacgtggacggcgtggaagtgcacaacgccaagaccaagcctagagaggaacagtacaacagcacctaccgggtggtgtccgtgctgacagtgctgcaccaggactggctgaacggcaaagagtacaagtgcaaggtgtccaacaaggccctgcctgcccccatcgagaaaaccatcagcaaggccaagggccagccccgcgaaccccaggtgtacacactgcccccaagcagggacgagctgaccaagaaccaggtgtccctgacctgtctcgtgaaaggcttctacccctccgatatcgccgtggaatgggagagcaacggccagcccgagaacaactacaagaccaccccccctgtgctggacagcgacggctcattcttcctgtacagcaagctgaccgtggacaagtcccggtggcagcagggcaacgtgttcagctgcagcgtgatgcacgaggccctgcacaaccactacacccagaagtccctgagcctgagccccggcaaatga

SEQ ID NO: 39 - DNA, 633 bp, Artificial Sequence
  Antibody light chain
tcgtatgagctgacacaacctccctcagtgtccgtaagtccaggacagactgcgagaatcacctgctctggaggcaatcgcaactactactatgggtggtatcagcagaaacccggacaagctcctgtgaccgtcatctatgccaacgacaaacggccatcaggcattccggagaggttcagcggtagcaattccgggtctaccaccactctcacgataagtggggttcaggctgaagatgaagccgactactactgtggcacagcatacacaggcaagtacgtgtttggtggaggcactaagctgacagtccttggtcagcccaaggctgccccctcggtcactctgttcccgccctcctctgaggagcttcaagccaacaaggccacactggtgtgtctcataagtgacttctacccgggagccgtgacagtggcctggaaggcagatagcagccccgtcaaggcgggagtggagaccaccacaccctccaaacaaagcaacaacaagtacgcggccagcagctatctgagcctgacgcctgagcagtggaagtcccacagaagctacagctgccaggtcacgcatgaagggagcaccgtggagaagacagtggcccctacagaatgttag

SEQ ID NO: 40 - DNA, 1353 bp, Artificial Sequence
  Antibody heavy chain
gaggtgcagctgttggagtctgggggaggactggtgcagcctggcggaagcctgagactgtcttgtgccgccagcggcttcaccttcagcacctatgccatgggctgggtgcgccaggcccctggaaagggcctggaatttgtggccgccatccggaacgatggcagctggacaggatatggcgccgctgtgaagggccggttcaccatcagccgggacaacagcaagaacaccctgtacctgcagatgagcagcctgcgggccgaggacaccgccgtgtactactgtgccaagtacaccggcagcagcggcggctctattggagcttggggacagggaaccctggtcaccgtctcctcagcctctacaaagggccccagcgtgttccctctggcccctagcagcaagagcacatctggcggaacagccgccctgggctgcctcgtgaaggactactttcccgagcccgtgaccgtgtcctggaactctggcgctctgacaagcggcgtgcacacctttccagccgtgctgcagagcagcggcctgtactctctgagcagcgtcgtgacagtgcccagcagctctctgggcacccagacctacatctgcaacgtgaaccacaagcccagcaacaccaaggtggacaagaaggtggaacccaagagctgcgacaagacccacacctgtcccccttgtcctgcccccgaactgctgggaggcccttccgtgttcctgttccccccaaagcccaaggacaccctgatgatcagccggacccccgaagtgacctgcgtggtggtggatgtgtcccacgaggaccctgaagtgaagttcaattggtacgtggacggcgtggaagtgcacaacgccaagaccaagcctagagaggaacagtacaacagcacctaccgggtggtgtccgtgctgacagtgctgcaccaggactggctgaacggcaaagagtacaagtgcaaggtgtccaacaaggccctgcctgcccccatcgagaaaaccatcagcaaggccaagggccagccccgcgaaccccaggtgtacacactgcccccaagcagggacgagctgaccaagaaccaggtgtccctgacctgtctcgtgaaaggcttctacccctccgatatcgccgtggaatgggagagcaacggccagcccgagaacaactacaagaccaccccccctgtgctggacagcgacggctcattcttcctgtacagcaagctgaccgtggacaagtcccggtggcagcagggcaacgtgttcagctgcagcgtgatgcacgaggccctgcacaaccactacacccagaagtccctgagcctgagccccggcaaatga